European Patent Application EP 4 234 671 A1, published August 30, 2023. Title: Compositions containing biosurfactants and a lipase from Stachybotrys chlorohalonata. Applicant: Evonik Operations GmbH. The sequence listing filed with the application follows.

SEQUENCE LISTING (2 sequences)

SEQ ID NO: 1 - protein, 347 aa, Stachybotrys chlorohalonata
MLGYILLSFAALAAAAPLSATDYVNAFKARSLDGRAAVTEQVLADFRIYAEYAGAAYCNSEVAPGTAITCGGSAGPCPSVEGNAATVLQSFEGLLTGIGGYVAVDHARSEIIISIRGSNNLRNFLTDVVFIRQGCDLFSGCQVHAGFGTAWKEIESRATAAVAAAVAANPGYSVVATGHSLGGAVATIAAGYLRRSHAVDIYTFGAPRVGNAAFSQFITDQAGGEFRVTHVDDPVPRLPPMIFGYRHISPEYWLSTGDGENLEFAVGDVIVCQGISTTGCNAGTNVGLNIPAHLNYIVEISSCGPAFSFRQASEVSNEDLAVRLHEWALADQEYAAAINGAAAAPAA

SEQ ID NO: 2 - DNA, 1044 bp, synthetic construct
  misc_feature 1..1044: note = CodonOpimized for P. pastoris
  source 1..1044: mol_type = other DNA
atgttgggttacatactgttgagttttgctgctttagctgcagctgctccattatctgccacagactatgtcaatgccttcaaagctagatccttggacggtagagcagccgttacagaacaagtgcttgctgattttaggatatatgctgaatacgccggtgcagcatactgcaattccgaggttgctccaggcaccgctataacctgcggtggaagtgcaggcccttgtcccagtgttgagggtaacgccgccactgttctgcagtcatttgagggtctgcttaccggaatcggaggttatgtagcagttgaccatgctcgaagtgaaattatcatctcaattagaggttccaacaaccttagaaacttcttgactgatgtggtttttattagacagggatgcgacctattttctggatgtcaagttcacgccggatttggtaccgcttggaaggaaatcgaatccagggctactgcagcagtggcagccgcagtagcagccaacccaggttattctgtcgttgccactggtcactcacttggtggcgcagttgctactattgcagccggatatttgagacgatcacatgcagtcgatatatacacattcggagcaccaagagtcggtaacgcagctttctcccagtttataacagaccaggctggtggagagtttagagttactcatgtagatgaccctgtgcctcgtttaccaccaatgatattcggatacagacacatttctcctgagtactggcttagtacgggagacggtgaaaatttggaatttgctgttggcgacgtcattgtgtgtcagggtatttcaactacaggttgcaatgccggcactaacgtcggcttgaatatccctgctcacttgaactacatagtggaaatttctagttgtggccctgccttcagttttagacaagcttcagaggttagtaatgaggatctggcagtaagattgcacgagtgggctctagcagatcaagaatacgctgcagccattaacggagccgctgctgcaccagctgcatga